European Patent Application EP 4 786 582 A1, published August 5, 2026. Title: HLA gene-modified cell. Applicant: Ajinomoto Co., Inc. The sequence listing filed with the application follows.

SEQUENCE LISTING (11 sequences)

SEQ ID NO: 1 - protein, 448 aa, synthetic construct
  source 1..448: note = Single Chain Dimer (SCD)
MSRSVALAVLALLSLSGLEAIQRTPKIQVYSRHPAENGKSNFLNCYVSGFHPSDIEVDLLKNGERIEKVEHSDLSFSKDWSFYLLYYTEFTPTEKDEYACRVNHVTLSQPKIVKWDRDMGGGGSGGGGSGGGGSGSHSMRYFSAAVSRPGRGEPRFIAMGYVDDTQFVRFDSDSACPRMEPRAPWVEQEGPEYWEEETRNTKAHAQTDRMNLQTLRGYYNQSEASSHTLQWMIGCDLGSDGRLLRGYEQYAYDGKDYLALNEDLRSWTAADTAAQISKRKCEAANVAEQRRAYLEGTCVEWLHRYLENGKEMLQRADPPKTHVTHHPVFDYEATLRCWALGFYPAEIILTWQRDGEDQTQDVELVETRPAGDGTFQKWAAVVVPSGEEQRYTCHVQHEGLPEPLMLRWKQSSLPTIPIMGIVAGLVVLAAVVTGAAVAAVLWRKKSSD

SEQ ID NO: 2 - DNA, 1347 bp, synthetic construct
  source 1..1347: mol_type = other DNA; note = Single Chain Dimer (SCD)
atgtctcgctccgtggccttagctgtgctcgcgctactctctctttctggcctggaggctatccagcgtactccaaagattcaggtttactcacgtcatccagcagagaatggaaagtcaaatttcctgaattgctatgtgtctgggtttcatccatccgacattgaagttgacttactgaagaatggagagagaattgaaaaagtggagcattcagacttgtctttcagcaaggactggtctttctatctcttgtactacactgaattcacccccactgaaaaagatgagtatgcctgccgtgtgaaccatgtgactttgtcacagcccaagatagttaagtgggatcgagacatgggtggtggcggatccggtggtggcggttctggtggtggcggctccggctcccactccatgaggtatttcagcgccgccgtgtcccggcccggccgcggggagccccgcttcatcgccatgggctacgtggacgacacgcagttcgtgcggttcgacagcgactcggcgtgtccgaggatggagccgcgggcgccgtgggtggagcaggaggggccggagtattgggaagaggagacacggaacaccaaggcccacgcacagactgacagaatgaacctgcagaccctgcgcggctactacaaccagagcgaggccagttctcacaccctccagtggatgattggctgcgacctggggtccgacggacgcctcctccgcgggtatgaacagtatgcctacgatggcaaggattacctcgccctgaacgaggacctgcgctcctggaccgcagcggacactgcggctcagatctccaagcgcaagtgtgaggcggccaatgtggctgaacaaaggagagcctacctggagggcacgtgcgtggagtggctccacagatacctggagaacgggaaggagatgctgcagcgcgcggacccccccaagacacacgtgacccaccaccctgtctttgactatgaggccaccctgaggtgctgggccctgggcttctaccctgcggagatcatactgacctggcagcgggatggggaggaccagacccaggacgtggagctcgtggagaccaggcctgcaggggatggaaccttccagaagtgggcagctgtggtggtgccttctggagaggagcagagatacacgtgccatgtgcagcatgaggggctgccggagcccctcatgctgagatggaagcagtcttccctgcccaccatccccatcatgggtatcgttgctggcctggttgtccttgcagctgtagtcactggagctgcggtcgctgctgtgctgtggagaaagaagagctcagattga

SEQ ID NO: 3 - protein, 15 aa, synthetic construct
  source 1..15: note = linker between B2M and HLA-G alpha chain
GGGGSGGGGSGGGGS

SEQ ID NO: 4 - protein, 477 aa, synthetic construct
  source 1..477: note = Single Chain Dimer (SCD)
MSRSVALAVLALLSLSGLEAIQRTPKIQVYSRHPAENGKSNFLNCYVSGFHPSDIEVDLLKNGERIEKVEHSDLSFSKDWSFYLLYYTEFTPTEKDEYACRVNHVTLSQPKIVKWDRDMGGGGSGGGGSGGGGSMKTPRMVVMAPRTLFLLLSGALTLTETWAGSHSMRYFSAAVSRPGRGEPRFIAMGYVDDTQFVRFDSDSACPRMEPRAPWVEQEGPEYWEEETRNTKAHAQTDRMNLQTLRGYYNQSEASSHTLQWMIGCDLGSDGRLLRGYEQYAYDGKDYLALNEDLRSWTAADTAAQISKRKCEAANVAEQRRAYLEGTCVEWLHRYLENGKEMLQRADPPKTHVTHHPVFDYEATLRCWALGFYPAEIILTWQRDGEDQTQDVELVETRPAGDGTFQKWAAVVVPSGEEQRYTCHVQHEGLPEPLMLRWKQSSLPTIPIMGIVAGLVVLAAVVTGAAVAAVLWRKKSSD

SEQ ID NO: 5 - DNA, 1434 bp, synthetic construct
  source 1..1434: mol_type = other DNA; note = Single Chain Dimer (SCD)
atgtctcgctccgtggccttagctgtgctcgcgctactctctctttctggcctggaggctatccagcgtactccaaagattcaggtttactcacgtcatccagcagagaatggaaagtcaaatttcctgaattgctatgtgtctgggtttcatccatccgacattgaagttgacttactgaagaatggagagagaattgaaaaagtggagcattcagacttgtctttcagcaaggactggtctttctatctcttgtactacactgaattcacccccactgaaaaagatgagtatgcctgccgtgtgaaccatgtgactttgtcacagcccaagatagttaagtgggatcgagacatgggtggtggcggatccggtggtggcggttctggtggtggcggctccatgaagacgccaaggatggtggtcatggcgccccgaaccctcttcctgctgctctcgggggccctgaccctgaccgagacctgggcgggctcccactccatgaggtatttcagcgccgccgtgtcccggcccggccgcggggagccccgcttcatcgccatgggctacgtggacgacacgcagttcgtgcggttcgacagcgactcggcgtgtccgaggatggagccgcgggcgccgtgggtggagcaggaggggccggagtattgggaagaggagacacggaacaccaaggcccacgcacagactgacagaatgaacctgcagaccctgcgcggctactacaaccagagcgaggccagttctcacaccctccagtggatgattggctgcgacctggggtccgacggacgcctcctccgcgggtatgaacagtatgcctacgatggcaaggattacctcgccctgaacgaggacctgcgctcctggaccgcagcggacactgcggctcagatctccaagcgcaagtgtgaggcggccaatgtggctgaacaaaggagagcctacctggagggcacgtgcgtggagtggctccacagatacctggagaacgggaaggagatgctgcagcgcgcggacccccccaagacacacgtgacccaccaccctgtctttgactatgaggccaccctgaggtgctgggccctgggcttctaccctgcggagatcatactgacctggcagcgggatggggaggaccagacccaggacgtggagctcgtggagaccaggcctgcaggggatggaaccttccagaagtgggcagctgtggtggtgccttctggagaggagcagagatacacgtgccatgtgcagcatgaggggctgccggagcccctcatgctgagatggaagcagtcttccctgcccaccatccccatcatgggtatcgttgctggcctggttgtccttgcagctgtagtcactggagctgcggtcgctgctgtgctgtggagaaagaagagctcagattga

SEQ ID NO: 6 - protein, 500 aa, synthetic construct
  source 1..500: note = Single Chain Trimer (SCT)
MSRSVALAVLALLSLSGLEAVMAPRTLFLGGGGSGGGGSGGGGSIQRTPKIQVYSRHPAENGKSNFLNCYVSGFHPSDIEVDLLKNGERIEKVEHSDLSFSKDWSFYLLYYTEFTPTEKDEYACRVNHVTLSQPKIVKWDRDMGGGGSGGGGSGGGGSGGGGSGSHSLKYFHTSVSRPGRGEPRFISVGYVDDTQFVRFDNDAASPRMVPRAPWMEQEGSEYWDRETRSARDTAQIFRVNLRTLRGYYNQSEAGSHTLQWMHGCELGPDGRFLRGYEQFAYDGKDYLTLNEDLRSWTAVDTAAQISEQKSNDASEAEHQRAYLEDTCVEWLHKYLEKGKETLLHLEPPKTHVTHHPISDHEATLRCWALGFYPAEITLTWQQDGEGHTQDTELVETRPAGDGTFQKWAAVVVPSGEEQRYTCHVQHEGLPEPVTLRWKPASQPTIPIVGIIAGLVLLGSVVSGAVVAAVIWRKKSSGGKGGSYSKAEWSDSAQGSESHSL

SEQ ID NO: 7 - DNA, 1503 bp, synthetic construct
  source 1..1503: mol_type = other DNA; note = Single Chain Trimer (SCT)
atgtctcgctccgtggccttagctgtgctcgcgctactctctctttctggcctggaggctgtcatggcgccccgaaccctcttcctgggtggtggcggatccggtggtggcggttctggtggtggcggctccatccagcgtactccaaagattcaggtttactcacgtcatccagcagagaatggaaagtcaaatttcctgaattgctatgtgtctgggtttcatccatccgacattgaagttgacttactgaagaatggagagagaattgaaaaagtggagcattcagacttgtctttcagcaaggactggtctttctatctcttgtactacactgaattcacccccactgaaaaagatgagtatgcctgccgtgtgaaccatgtgactttgtcacagcccaagatagttaagtgggatcgagacatgggtggtggcggttctggtggtggcggtagtggcggcggaggaagcggtggtggcggttccggctcccactccttgaagtatttccacacttccgtgtcccggcccggccgcggggagccccgcttcatctctgtgggctacgtggacgacacccagttcgtgcgcttcgacaacgacgccgcgagtccgaggatggtgccgcgggcgccgtggatggagcaggaggggtcagagtattgggaccgggagacacggagcgccagggacaccgcacagattttccgagtgaatctgcggacgctgcgcggctactacaatcagagcgaggccgggtctcacaccctgcagtggatgcatggctgcgagctggggcccgacgggcgcttcctccgcgggtatgaacagttcgcctacgacggcaaggattatctcaccctgaatgaggacctgcgctcctggaccgcggtggacacggcggctcagatctccgagcaaaagtcaaatgatgcctctgaggcggagcaccagagagcctacctggaagacacatgcgtggagtggctccacaaatacctggagaaggggaaggagacgctgcttcacctggagcccccaaagacacacgtgactcaccaccccatctctgaccatgaggccaccctgaggtgctgggccctgggcttctaccctgcggagatcacactgacctggcagcaggatggggagggccatacccaggacacggagctcgtggagaccaggcctgcaggggatggaaccttccagaagtgggcagctgtggtggtgccttctggagaggagcagagatacacgtgccatgtgcagcatgaggggctacccgagcccgtcaccctgagatggaagccggcttcccagcccaccatccccatcgtgggcatcattgctggcctggttctccttggatctgtggtctctggagctgtggttgctgctgtgatatggaggaagaagagctcaggtggaaaaggagggagctactctaaggctgagtggagcgacagtgcccaggggtctgagtctcacagcttgtaa

SEQ ID NO: 8 - DNA, 15 bp, synthetic construct
  source 1..15: mol_type = other DNA; note = linker between signal peptide and B2M
ggggsggggsggggs

SEQ ID NO: 9 - DNA, 15 bp, synthetic construct
  source 1..15: mol_type = other DNA; note = linker between B2M and HLA-E alpha chain
ggggsggggsggggs

SEQ ID NO: 10 - DNA, 4050 bp, synthetic construct
  source 1..4050: mol_type = other DNA; note = HLA-A alpha chain gene promoter
aagacaagcttaaagagttaatgaaaaataattagatacaagaagactttgattttcagaaacctgaaacaatagttataattttgcttttaacgtatattcaaatcctttgatactgttcctttctagaggtgcagcttaattccctctcttgagtgtggcttggacttaatgaggcacttctgaaatggcctggttctgtgttcccacccaaatctcatcttgaattgttatgcaaattgtaatccctacctattgggggagggacctcatgggaggtgattggatcatggggacggtgcccccatgctgttctcctgatgctgagggaattctcatgagatctgatggttttataaggggcttttccctgcttcattgtgcatttctctctcctgtcaccacgtgaagaaggacgggtttgcttccacttctgccgtgactgtaagtttcctggggcagcctcctcagtcatgcagaactgtgagtcaattaaatctctttcctttataaattacccagtctcatgtatttctttatagcagtgtgagaatggactaatacaacttctaacttatagaatagtgccaacataacagtttgtgactctgggtgtagaacataaaactaactgcggcttccaccttctctctctctgaatctgggatcatgagctctgggggaagccagccgctctgccataagcagccctgcaggaaggtccacatgactgagaactgaggccttctgggaacagacaacaaggaaccaggccttttccaacagccatgtgactgatccatgtttcttgtgaattcccagccccagcgaagcccttggatgctgcggcccctggctgacaactggagtgcagccttttgagaggccctgagcaggaagcactcagggaaacctttcctggattcctgacgattggaaactgtgggagatgagaaacatttgttgtttcgagctaagttttacgtaatttgttatgcaatagtaaataatatattttcacaagagaagatgtattattacacatcaaattgcatttgctctaaatgtgtcatcatcatcattattatttttgagacagggtcttgctctgtcacccaggctggaatgcagtggcatgatcaccatgcactgcagtgtcgaacgcctggggtcaagggactctctgacctcagcctcctgagtagctgcgactaccatcatgaactaccatgcctggctaattttctaattttttgtagagatggaggttttgcccaggttgatcttgaacttctggagtcaacaaatctcccttactccaccttccacagtgctatgatgacaggcgtgagccaccatacctggcctaaattaattataagatattaaacatgtaacttagttttaaaaggtaaggacaatttccatggctgaagaggatgtattttatgaccgttcacaatgatcactttacttgaacttcactttccaactgtgtcccaattaaacacaaaaggaagatccaacccttgctaggctgattctatgaaggcctcaacaagcagctcctggtcattcaccttcctccagttattcaaccaactctaatataggtgctgctgtgaagggatttagcagatataattaagggtctcaattagttgatttatgctgggtttatcctgcttgaactgtcctaatcaggtgagcccttgaaaggactgggttcttcatgagcatagagacttacagtgtgagagggactcagcatgaggggtttcctccaccatgggctttgaaaaggaaagggctatgggccgggcgcggtggctcacgcctgtaatcccgacactttgggaggccgaggcgggtggatcatgaggtcaggaggttgagacaatcctggctaacaaggtgaaaccctgtctctactaagaaaaaaaaaaaaaattagcagagtgtagtggtgggcacctgtagtctcagctacttgggactgagacaggagaatggtgtgaacccaggaggtggagcttgtagtgagcagagatcattgggccactgtaccccagcctgggctacagagccagactccgtctcaaaaaaaaaaaaaaaaaaaaaaaaaaaattaaggggctgtgtaggaaagaatgctggtgagcaccgggaattgagcccctcccagttctctacactgacagctagccaggaacagggacctcagtctttacaactgccaaaaactgcattccgccacctctgtataaacctgaaggaggattcaaaatgaaaacacagcttttggaagcccagaacagagattctatccacatcttgcccagatttctgaccaaggaactataagcagataaatgggtgttgtttcgccaggcgtggtagtgtgcgaatgaattgatatacacactagttgcataaaataaaatctttctgaactttttcagtgttttacagtttataattatctgtgatgcaatttaatacactcatatttcattcattaaatcaacaaaaattaacttagtccctacaatgaaccaggtatcccctcatatgctcaagtgcctgacactccagaagcttcacaagaccgaggtggagacactggagtgttttaagtggagaaataacacactccgactcacaggagcaggaccactgtgaaaaaaacagttacgtagcaggtcatgggacagtgctagtgtcacaattcatgagtgacagtgtggtggggactaaggggacaggagggcctgaaggatgagaaggacggagggaagggctggagaagcaggaggtgaggaaaaggagcagaggaaagaatttgaaagcagcagaattcttaggtttaaatacattgttttatggattttaatacatccatctacagagcctagcagggtgtccttggcagttgtcttttaatacctcatgtgggtctgcctaaaaactaattttttatgttaatcaggtttaaaaaatactaagtgttcctataaaatatacacaacacttagaagtggatacttcctaaaaacagacagtgcatgagcactagtgaggggcattgtgagtgcattgaacagttgcaactttgaggtgaataaagcctgtaatggcttctggttgcaacatataggaacacagtcgctactttgtattgaggagatgtcctggactcacacagaaactcagagctatggaatgatggtaaatttaaaatactacaagcaggagtcacagatacattgtctgggaaaatgcaacttagtagctttgtgagtcctgttgtaaggcttttggacacatttatacatcaaggggccaaagtcacattttttacctattagattcctgatcattcaggggttaccaagattctgctacccactgtagttaataaacaaagagcaaattggtctctattctgtctcatgcactcaggcgcaactcttcccgattaaaaacaaaaacaacaacaacaaaaatctacacctccattcccagagcaagcttactctctggcaccaaactccatgggatgatttttcttctagaagagtccaggtggacaggtaaggagtgggagtcagggagtccagttcagggacagagattacgggataaaaagtgaaaggagagggacggggcccatgccgagggtttctcccttgtttctcagacagctcttgggccaagactcagggagacattgagacagagcgcttggcacagaagcagaggggtcagggcgaagtcccagggccccaggcgtggctctcagggtctcaggccccgaaggcggtgtatggattggggagtcccagccttggggattccccaactccgcagtttcttttctccctctcccaacctatgtagggtccttcttcctggatactcacgacgcggacccagttctcactcccattgggtgtcgggtttccagagaagccaatcagtgtcgtcgcggtcgcggttctaaagtccgcacgcacccaccgggactcagattctccccagacgccgagg

SEQ ID NO: 11 - DNA, 2473 bp, synthetic construct
  source 1..2473: mol_type = other DNA; note = HLA-B alpha chain gene promoter
agctgtgagagacacatcagagccctgggcactgtcgctgcctggagtagaacaaaaacaggacctggtcagagcccgcaggagacgtgggacaggaggaattatggggtgggtgagctcctccacactcccacccccaccacttacacgcagcctgagagtagctccctccttttccacctgtgggaagaaaatgtcctgtgagggcactgggaggaagcagggccatgagatcttagaggaacctcctagtcttggacccaaaaggaatttccagaagtatgactacagacccagggcaggatcaggaaacacgaggaaagcaagtgtgggtcctggaccaactgccctcctaaggtctgtccttagcagggaccttcccctgactcatgaatgctggaatcaggaccccaacaccacaaccatcaaggtgatacatccatccttcattgtcacatgtgctgcacaaaagagtaagtgctggcacacagggtcccaggctgcgttagcccctgtgtgcatgctgcttcccagtaatgaggcagggaacacttctacctggggcttgaaacccccagtgggacaagaaaacccagaccccacccctcaccccttccctacctgaactcttcctcctacacatcacagcagcgaccacagctccgatgaccacaactgctaggacagccaggccagcaacaatgcccacgatggggacggtggactgggaagacggctctgggaaaggaggggaagatgaggggccctgaccctgctgaagggctcctgctttccctgagaagagatatgacccctcatccccctccttaccccatctcagggtgaggggcttcggcagcccctcatgctgtacatggcatgtgtatctctgctcttctccagaaggcaccaccacagctgcccacttctggaaggttctatctcctgctggtctggtctccacaagctcagtgtcctgagtttggtcctcgccatcccgctgccaggtcagtgtgatctccgcagggtagaaacccagggcccagcacctcagggtggcctcatggtcagagatggggtggtgggtcacgtgtgtctttggggggtctgatgggaagagtcagaaaattcaggcgctttgcatctttcatgggacaccctaggaccacccatgtgaccagcctgagaatggacaggacacctggggtggggaaggggcacagaacccagacaccagcctggacgcaggcacctgggataatctcctattcattggaaagttcgagtctctgagcggggaacagggacttctgctcctgatctgagtggaggtaaagtgactcagaagtgctggaatcagagccccaaacacactgagtgtgaggcagagaacaaggcctgagaggaaaagtcacggttcccaaggctgctgcaggggtcaaaggggacccctgatcagtattctagggactgtcttcccctccatttcctcagagacgtcattccttaattgtctagagagaagagggggccctcagaggaaactcaggaaaactcatgccattctccattcaacggagggcgacattctagcgctgatcccattttcctcctcttctcgtgggaggccatccccggcgacctataggagatggggaaggctccccactgcccctggtaccagcgcgctccagcttgtccttcccgttctccaggtatctgcggagccactccacgcactcgccctccaggtaggctctccgctgctccgcctcacgggccgcctcccacttgcgctgggtgatctgagccgccgtgtccgcggcggtccaggagcgcaggtcctcgttcagggcgatgtaatccttgccgtcgtaggcgtactggtcatgcccgcggaggaggcgcccgtccggccccacgtcgcagccgtacatgctctggagggtgtgagaccctggccccggccccgcggtcagcccagtcccccgagccccgccccgccccgaccaacccgcggggattttggcctcaactgaaaatgaaaccgggtaaacgcgcctggggctctcgccggtcgagggtctgggcgggtcccgcggcctcagggaggcggatctcggacccggagactcggggcgacccgggccgtacgtgggggatggggagtcgtgacctgcgccccgggccggggtcactcaccggcctcgctctggttgtagtagccgcgcaggttccgcaggctctctcggtcagtctgtgcctgggccttgtagatctgtgtgttccggtcccaatactccggcccctcctgctctatccacggcgcccgcggctcctctctcggactcgcggcgtcgctgtcgaacctcacgaactgggtgtcgtccacgtagcccactgagatgaagcggggctccccgcggccgggccgggacacggaggtgtagaaatacctcatggagtgggagcc